European Patent Application EP 4 349 983 A1, published April 10, 2024. Title: Method for editing genome. Applicant: NATIONAL INSTITUTE OF ADVANCED INDUSTRIAL SCIENCE AND TECHNOLOGY. The sequence listing filed with the application follows.

SEQUENCE LISTING (27 sequences)

SEQ ID NO: 1 - DNA, 101 bp, Artificial Sequence
  synthesized polynucleotide
tgtcctccctgcctggcggcccccttctcctggtcccggcgctggggacgctgcttccccatcgccgagttaggcaggacccggagccggtgcgaatcctg

SEQ ID NO: 2 - DNA, 81 bp, Artificial Sequence
  synthesized polynucleotide
gcctggcggcccccttctcctggtcccggcgctggggacgctgcttccccatcgccgagttaggcaggacccggagccggt

SEQ ID NO: 3 - DNA, 130 bp, Artificial Sequence
  synthesized polynucleotide
agggaggacagcggttcccgaggaaggtttcggagagtgaaagagaccggaggggaggcggctgatgtccacgcccgagccaagactctcaaatcccacatcaatttcccgaggcgactctcgcaatcgc

SEQ ID NO: 4 - DNA, 130 bp, Artificial Sequence
  synthesized polynucleotide
ctctatcaggaaaatcaaattaaacaagcctttccttcctggttccactcgccaaggattcgacatcggggttgttggtttaacttcccttttccccagaggcgcttcgctgtcaggccccaggattcgc

SEQ ID NO: 5 - DNA, 120 bp, Artificial Sequence
  synthesized polynucleotide
gcggttcccgaggaaggtttcggagagtgaaagagaccggaggggaggcggctgatgtccacgcccgagccaagactctcaaatcccacatcaatttcccgaggcgactctcgcaatcgc

SEQ ID NO: 6 - DNA, 120 bp, Artificial Sequence
  synthesized polynucleotide
ctctatcaggaaaatcaaattaaacaagcctttccttcctggttccactcgccaaggattcgacatcggggttgttggtttaacttcccttttccccagaggcgcttcgctgtcaggccc

SEQ ID NO: 7 - DNA, 10 bp, Artificial Sequence
  synthesized polynucleotide
agggaggaca

SEQ ID NO: 8 - DNA, 10 bp, Artificial Sequence
  synthesized polynucleotide
caggattcgc

SEQ ID NO: 9 - DNA, 130 bp, Artificial Sequence
  synthesized polynucleotide
gccgccaggcagggaggacagcggttcccgaggaaggtttcggagagtgaaagagaccggaggggaggcggctgatgtccacgcccgagccaagactctcaaatcccacatcaatttcccgaggcgactc

SEQ ID NO: 10 - DNA, 130 bp, Artificial Sequence
  synthesized polynucleotide
aaaatcaaattaaacaagcctttccttcctggttccactcgccaaggattcgacatcggggttgttggtttaacttcccttttccccagaggcgcttcgctgtcaggccccaggattcgcaccggctccg

SEQ ID NO: 11 - DNA, 100 bp, Artificial Sequence
  synthesized polynucleotide
agggaggacagcggttcccgaggaaggtttcggagagtgaaagagaccggaggggaggcggctgatgtccacgcccgagccaagactctcaaatcccaca

SEQ ID NO: 12 - DNA, 100 bp, Artificial Sequence
  synthesized polynucleotide
tttccttcctggttccactcgccaaggattcgacatcggggttgttggtttaacttcccttttccccagaggcgcttcgctgtcaggccccaggattcgc

SEQ ID NO: 13 - DNA, 70 bp, Artificial Sequence
  synthesized polynucleotide
agggaggacagcggttcccgaggaaggtttcggagagtgaaagagaccggaggggaggcggctgatgtcc

SEQ ID NO: 14 - DNA, 70 bp, Artificial Sequence
  synthesized polynucleotide
cgacatcggggttgttggtttaacttcccttttccccagaggcgcttcgctgtcaggccccaggattcgc

SEQ ID NO: 15 - DNA, 40 bp, Artificial Sequence
  synthesized polynucleotide
agggaggacagcggttcccgaggaaggtttcggagagtga

SEQ ID NO: 16 - DNA, 40 bp, Artificial Sequence
  synthesized polynucleotide
tttccccagaggcgcttcgctgtcaggccccaggattcgc

SEQ ID NO: 17 - DNA, 103 bp, Artificial Sequence
  synthesized polynucleotide
tgtcctccctgcctggcggcccccttctcctggtcccggcgctggggacgtgctgcttccccatcgccgagttaggcaggacccggagccggtgcgaatcctg

SEQ ID NO: 18 - DNA, 98 bp, Artificial Sequence
  synthesized polynucleotide
tgtcctccctgcctggcggcccccttctcctggtcccggcgctggggacgcttccccatcgccgagttaggcaggacccggagccggtgcgaatcctg

SEQ ID NO: 19 - DNA, 101 bp, Artificial Sequence
  synthesized polynucleotide
aggtcaagatggaagaaatcctgaggaagctgcagaaggaggcgtccgggcgcaagtacaaagccatcaaggagagctgcacctgggccctgggtaagcgt

SEQ ID NO: 20 - DNA, 130 bp, Artificial Sequence
  synthesized polynucleotide
atcttgaccttccaggcgccgggccgccgcccacagggagagaagcgcgggcgagccgggccggggaagccgccgctgcctggccctgggcgcctaggcggccgccgcgcgcgcccccatgccgccccgg

SEQ ID NO: 21 - DNA, 130 bp, Artificial Sequence
  synthesized polynucleotide
ggcgactctcgcaatcgccagaacggcacccatgaccgacgctccgcgaaagccccacgcgcggaggcgcgggttcagccccggccgcgcggccctcccgccgcggcgagcaggtgccggacgcttaccc

SEQ ID NO: 22 - DNA, 80 bp, Artificial Sequence
  synthesized polynucleotide
agggaggacagcggttcccgaggaaggtttcggagagtgaaagagaccggaggggaggcggctgatgtccacgcccgagc

SEQ ID NO: 23 - DNA, 80 bp, Artificial Sequence
  synthesized polynucleotide
gccaaggattcgacatcggggttgttggtttaacttcccttttccccagaggcgcttcgctgtcaggccccaggattcgc

SEQ ID NO: 24 - DNA, 60 bp, Artificial Sequence
  synthesized polynucleotide
agggaggacagcggttcccgaggaaggtttcggagagtgaaagagaccggaggggaggcg

SEQ ID NO: 25 - DNA, 60 bp, Artificial Sequence
  synthesized polynucleotide
gttgttggtttaacttcccttttccccagaggcgcttcgctgtcaggccccaggattcgc

SEQ ID NO: 26 - DNA, 50 bp, Artificial Sequence
  synthesized polynucleotide
agggaggacagcggttcccgaggaaggtttcggagagtgaaagagaccgg

SEQ ID NO: 27 - DNA, 50 bp, Artificial Sequence
  synthesized polynucleotide
taacttcccttttccccagaggcgcttcgctgtcaggccccaggattcgc